European Patent Application EP 4 130 042 A1, published February 8, 2023. Title: 结合CD47的抗原结合多肽及用途. Applicant: 正大天晴药业集团股份有限公司. The sequence listing filed with the application follows.

SEQUENCE LISTING (198 sequences)

SEQ ID NO: 1 - protein, 10 aa, Mus musculus
GFSLTNYGVH

SEQ ID NO: 2 - protein, 10 aa, Mus musculus
GFTFSNYYMS

SEQ ID NO: 3 - protein, 10 aa, Mus musculus
GYTFTNYGMN

SEQ ID NO: 4 - protein, 10 aa, Mus musculus
GYTFSRYWIE

SEQ ID NO: 5 - protein, 10 aa, Mus musculus
GFNIEDDYIE

SEQ ID NO: 6 - protein, 9 aa, Mus musculus
IIWAGGSTN

SEQ ID NO: 7 - protein, 10 aa, Mus musculus
YISSGGGSTY

SEQ ID NO: 8 - protein, 10 aa, Mus musculus
WINTNTGEPT

SEQ ID NO: 9 - protein, 8 aa, Mus musculus
EFIPGSDT

SEQ ID NO: 10 - protein, 10 aa, Mus musculus
RIDPANDKTK

SEQ ID NO: 11 - protein, 8 aa, Mus musculus
DDYASMDY

SEQ ID NO: 12 - protein, 3 aa, Mus musculus
FAY

SEQ ID NO: 13 - protein, 10 aa, Mus musculus
FSHLRGPMDY

SEQ ID NO: 14 - protein, 8 aa, Mus musculus
GGLRRMDY

SEQ ID NO: 15 - protein, 11 aa, Mus musculus
PGLRRYYSMDY

SEQ ID NO: 16 - protein, 16 aa, Mus musculus
RSSQSLVHSNGNTYLH

SEQ ID NO: 17 - protein, 16 aa, Mus musculus
KSSQSLLDSDGKTYLN

SEQ ID NO: 18 - protein, 16 aa, Mus musculus
RSSQSLVHSNGYTYLH

SEQ ID NO: 19 - protein, 12 aa, Mus musculus
RASSSVSSTYLH

SEQ ID NO: 20 - protein, 11 aa, Mus musculus
KASENVVSYVS

SEQ ID NO: 21 - protein, 7 aa, Mus musculus
KVSNRFS

SEQ ID NO: 22 - protein, 7 aa, Mus musculus
LVSKLDS

SEQ ID NO: 23 - protein, 7 aa, Mus musculus
KVSNRFS

SEQ ID NO: 24 - protein, 7 aa, Mus musculus
TTSTLAS

SEQ ID NO: 25 - protein, 7 aa, Mus musculus
GASNRYT

SEQ ID NO: 26 - protein, 9 aa, Mus musculus
SQSTHVPYT

SEQ ID NO: 27 - protein, 7 aa, Mus musculus
GTHFPLT

SEQ ID NO: 28 - protein, 9 aa, Mus musculus
SQSTHVPPT

SEQ ID NO: 29 - protein, 9 aa, Mus musculus
QQFSDSTWT

SEQ ID NO: 30 - protein, 9 aa, Mus musculus
GQSYSYPLT

SEQ ID NO: 31 - protein, 9 aa, 人工序列(Artificial Sequence)
QQFSESTWT

SEQ ID NO: 32 - protein, 9 aa, 人工序列(Artificial Sequence)
  UNSURE (5): Xaa is D or E
QQFSXSTWT

SEQ ID NO: 33 - protein, 116 aa, Mus musculus
QVQLKESGPGLVAPSQSLSITCTVSGFSLTNYGVHWVRQPPGKGLEWLGIIWAGGSTNYNSALMSRLSISKDNSKSQVFLKMNSLQTDDTAMYYCARDDYASMDYWGQGTSVTVSS

SEQ ID NO: 34 - protein, 112 aa, Mus musculus
DAFMTQTPLSLPVSLGDQASISCRSSQSLVHSNGNTYLHWYLQKPGQSPKLLIYKVSNRFSGVPDRFSGSGSGTDFTLKISRVEAEDLGVYFCSQSTHVPYTLGGGTKLEIK

SEQ ID NO: 35 - protein, 119 aa, Mus musculus
EVQLQQSGPELKKPGETVKISCKASGYTFTNYGMNWVKQVPGKGLKWMGWINTNTGEPTYAEEFKGRFAFSLETSARTAFLQINNLKNEDTATYFCTRFSHLRGPMDYWGQGASVTVSS

SEQ ID NO: 36 - protein, 112 aa, Mus musculus
DAVMTQTPLSLPVSLGDQASISCRSSQSLVHSNGYTYLHWYLQKPGQSPKLLIYKVSNRFSGVPDRFSGSGSGTDFTLKISRLEAEDLGVYFCSQSTHVPPTFGGGTKLEIK

SEQ ID NO: 37 - protein, 112 aa, Mus musculus
EVMLVESGGGLVQPGGSLKLSCAASGFTFSNYYMSWVRQTPEKRLEWVAYISSGGGSTYYPDSVKGRFTISRDNAKNTLYLQMSSLKSEDTAMYYCAWFAYWGQGTLVTVSA

SEQ ID NO: 38 - protein, 112 aa, Mus musculus
DAVVTQTPLTLSVTIGQPASISCKSSQSLLDSDGKTYLNWLLQRPGQSPKRLIYLVSKLDSGVPDRFTGSGSGTDFTLKISRVEAEDLGVYYCWQGTHFPLTFGAGTKLELK

SEQ ID NO: 39 - protein, 117 aa, Mus musculus
EVQLQQSVAELMKPGASVKIYCKATGYTFSRYWIEWVKQRPGHGLEWIGEFIPGSDTTNFNEKFKGKATFTAEISSNTAYMQLSSLTSEDSAVYFCARGGLRRMDYWGQGTSVTVSS

SEQ ID NO: 40 - protein, 108 aa, Mus musculus
DIVMTQTPAIMSASPGEKVTMTCRASSSVSSTYLHWYQQKSGASPKLWIYTTSTLASGVPARFSGSGSGTSYSLTISSVEAEDAATYYCQQFSDSTWTFGGGTKLEIK

SEQ ID NO: 41 - protein, 120 aa, Mus musculus
EVQLQQSGAEVARPGASVKLSCTVSGFNIEDDYIEWVKQRPEQGLEWIGRIDPANDKTKYAPKFQDKATITGDTSSNTAYLQLSSLTSEDTAVYYCTRPGLRRYYSMDYWGQGTSVTVSS

SEQ ID NO: 42 - protein, 107 aa, Mus musculus
NIVLTQSPKSMSMSVGERVTLSCKASENVVSYVSWYQQKPEQSPKLLIYGASNRYTGVPDRFIGSGSSTDFTLIISSFQPEDLADYHCGQSYSYPLTFGAGTKLELK

SEQ ID NO: 43 - protein, 117 aa, 人工序列(Artificial Sequence)
QVQLVQSGAEVKKPGSSVKVSCKASGYTFSRYWIEWVRQAPGQGLEWMGEFIPGSDTTNYAQKFQGRVTITADISTSTAYMELSSLRSEDTAVYYCARGGLRRMDYWGQGTLVTVSS

SEQ ID NO: 44 - protein, 108 aa, 人工序列(Artificial Sequence)
DIQMTQSPSSLSASVGDRVTITCRASSSVSSTYLHWYQQKPGKAPKLLIYTTSTLASGVPSRFSGSGSGTDFTLTISSLQPEDFATYYCQQFSDSTWTFGQGTKLEIK

SEQ ID NO: 45 - protein, 117 aa, 人工序列(Artificial Sequence); identical to SEQ ID NO: 43

SEQ ID NO: 46 - protein, 108 aa, 人工序列(Artificial Sequence)
DIQMTQSPSSLSASVGDRVTITCRASSSVSSTYLHWYQQKPGKAPKLLIYTTSTLASGVPSRFSGSGSGTDFTLTISSLQPEDFATYYCQQFSESTWTFGQGTKLEIK

SEQ ID NO: 47 - protein, 117 aa, 人工序列(Artificial Sequence); identical to SEQ ID NO: 43

SEQ ID NO: 48 - protein, 108 aa, 人工序列(Artificial Sequence)
DIQMTQSPSSLSASVGDRVTITCRASSSVSSTYLHWYQQKPGKAPKLLIYTTSTLASGVPSRFSGSGSGTSYTLTISSLQPEDFATYYCQQFSDSTWTFGQGTKLEIK

SEQ ID NO: 49 - protein, 117 aa, 人工序列(Artificial Sequence); identical to SEQ ID NO: 43

SEQ ID NO: 50 - protein, 108 aa, 人工序列(Artificial Sequence)
DIQMTQSPSSLSASVGDRVTITCRASSSVSSTYLHWYQQKPGKAPKLLIYTTSTLASGVPSRFSGSGSGTSYTLTISSLQPEDFATYYCQQFSESTWTFGQGTKLEIK

SEQ ID NO: 51 - protein, 117 aa, 人工序列(Artificial Sequence); identical to SEQ ID NO: 43

SEQ ID NO: 52 - protein, 108 aa, 人工序列(Artificial Sequence)
DIQMTQSPSSLSASVGDRVTITCRASSSVSSTYLHWYQQKPGKAPKLWIYTTSTLASGVPSRFSGSGSGTSYTLTISSLQPEDFATYYCQQFSDSTWTFGQGTKLEIK

SEQ ID NO: 53 - protein, 117 aa, 人工序列(Artificial Sequence); identical to SEQ ID NO: 43

SEQ ID NO: 54 - protein, 108 aa, 人工序列(Artificial Sequence)
DIQMTQSPSSLSASVGDRVTITCRASSSVSSTYLHWYQQKPGKAPKLWIYTTSTLASGVPSRFSGSGSGTSYTLTISSLQPEDFATYYCQQFSESTWTFGQGTKLEIK

SEQ ID NO: 55 - protein, 117 aa, 人工序列(Artificial Sequence)
QVQLVQSGAEVKKPGSSVKVSCKASGYTFSRYWIEWVRQAPGQGLEWMGEFIPGSDTTNYAQKFQGRVTITAEISTNTAYMELSSLRSEDTAVYYCARGGLRRMDYWGQGTLVTVSS

SEQ ID NO: 56 - protein, 108 aa, 人工序列(Artificial Sequence); identical to SEQ ID NO: 44

SEQ ID NO: 57 - protein, 117 aa, 人工序列(Artificial Sequence); identical to SEQ ID NO: 55

SEQ ID NO: 58 - protein, 108 aa, 人工序列(Artificial Sequence); identical to SEQ ID NO: 46

SEQ ID NO: 59 - protein, 117 aa, 人工序列(Artificial Sequence); identical to SEQ ID NO: 55

SEQ ID NO: 60 - protein, 108 aa, 人工序列(Artificial Sequence); identical to SEQ ID NO: 48

SEQ ID NO: 61 - protein, 117 aa, 人工序列(Artificial Sequence); identical to SEQ ID NO: 55

SEQ ID NO: 62 - protein, 108 aa, 人工序列(Artificial Sequence); identical to SEQ ID NO: 50

SEQ ID NO: 63 - protein, 117 aa, 人工序列(Artificial Sequence); identical to SEQ ID NO: 55

SEQ ID NO: 64 - protein, 108 aa, 人工序列(Artificial Sequence); identical to SEQ ID NO: 52

SEQ ID NO: 65 - protein, 117 aa, 人工序列(Artificial Sequence); identical to SEQ ID NO: 55

SEQ ID NO: 66 - protein, 108 aa, 人工序列(Artificial Sequence); identical to SEQ ID NO: 54

SEQ ID NO: 67 - protein, 119 aa, 人工序列(Artificial Sequence)
QVQLVQSGAEVKKPGASVKVSCKASGYTFTNYGMNWVRQAPGQGLEWMGWINTNTGEPTYAQKLQGRVTMTLDTSTRTAYMELRSLRSDDTAVYYCARFSHLRGPMDYWGQGTLVTVSS

SEQ ID NO: 68 - protein, 112 aa, 人工序列(Artificial Sequence)
DIQMTQSPSSLSASVGDRVTITCRSSQSLVHSNGYTYLHWYQQKPGKAPKLLIYKVSNRFSGVPSRFSGSGSGTDFTLTISSLQPEDFATYYCSQSTHVPPTFGQGTKLEIK

SEQ ID NO: 69 - protein, 119 aa, 人工序列(Artificial Sequence)
QVQLVQSGAEVKKPGASVKVSCKASGYTFTNYGMNWVRQAPGQGLKWMGWINTNTGEPTYAQELQGRVTMTLDTSTRTAYMELRSLRSDDTAVYYCTRFSHLRGPMDYWGQGTLVTVSS

SEQ ID NO: 70 - protein, 112 aa, 人工序列(Artificial Sequence); identical to SEQ ID NO: 68

SEQ ID NO: 71 - protein, 119 aa, 人工序列(Artificial Sequence)
QVQLVQSGAEVKKPGASVKVSCKASGYTFTNYGMNWVRQAPGQGLKWMGWINTNTGEPTYAQELQGRVTMTLDTSTRTAYMELRSLRSDDTAVYYCARFSHLRGPMDYWGQGTLVTVSS

SEQ ID NO: 72 - protein, 112 aa, 人工序列(Artificial Sequence); identical to SEQ ID NO: 68

SEQ ID NO: 73 - protein, 119 aa, 人工序列(Artificial Sequence); identical to SEQ ID NO: 71

SEQ ID NO: 74 - protein, 112 aa, 人工序列(Artificial Sequence)
DAQMTQSPSSLSASVGDRVTITCRSSQSLVHSNGYTYLHWYQQKPGKAPKLLIYKVSNRFSGVPSRFSGSGSGTDFTLTISSLQPEDFATYYCSQSTHVPPTFGQGTKLEIK

SEQ ID NO: 75 - protein, 119 aa, 人工序列(Artificial Sequence); identical to SEQ ID NO: 67

SEQ ID NO: 76 - protein, 112 aa, 人工序列(Artificial Sequence); identical to SEQ ID NO: 74

SEQ ID NO: 77 - protein, 119 aa, 人工序列(Artificial Sequence); identical to SEQ ID NO: 69

SEQ ID NO: 78 - protein, 112 aa, 人工序列(Artificial Sequence); identical to SEQ ID NO: 74

SEQ ID NO: 79 - protein, 120 aa, 人工序列(Artificial Sequence)
QVQLVQSGAEVKKPGASVKVSCKVSGFNIEDDYIEWVRQAPGQGLEWMGRIDPANDKTKYAQKFQGRVTMTGDTSTNTVYMELSSLRSEDTAVYYCARPGLRRYYSMDYWGQGTLVTVSS

SEQ ID NO: 80 - protein, 107 aa, 人工序列(Artificial Sequence)
DIQMTQSPSSLSASVGDRVTITCKASENVVSYVSWYQQKPGKAPKLLIYGASNRYTGVPSRFIGSGSSTDFTLTISSLQPEDFATYYCGQSYSYPLTFGQGTKLEIK

SEQ ID NO: 81 - protein, 120 aa, 人工序列(Artificial Sequence)
QVQLVQSGAEVKKPGASVKVSCKVSGFNIEDDYIEWVRQAPGQGLEWMGRIDPANDKTKYAQKFQGRVTMTGDTSTNTVYMELSSLRSEDTAVYYCTRPGLRRYYSMDYWGQGTLVTVSS

SEQ ID NO: 82 - protein, 107 aa, 人工序列(Artificial Sequence); identical to SEQ ID NO: 80

SEQ ID NO: 83 - protein, 117 aa, 人工序列(Artificial Sequence)
  UNSURE (73): Xaa is D or E
  UNSURE (74): Xaa is I or E
  UNSURE (77): Xaa is S or N
QVQLVQSGAEVKKPGSSVKVSCKASGYTFSRYWIEWVRQAPGQGLEWMGEFIPGSDTTNYAQKFQGRVTITAXXSTXTAYMELSSLRSEDTAVYYCARGGLRRMDYWGQGTLVTVSS

SEQ ID NO: 84 - protein, 108 aa, 人工序列(Artificial Sequence)
  UNSURE (48): Xaa is L or W
  UNSURE (71): Xaa is D or S
  UNSURE (72): Xaa is F or Y
  UNSURE (94): Xaa is D or E
DIQMTQSPSSLSASVGDRVTITCRASSSVSSTYLHWYQQKPGKAPKLXIYTTSTLASGVPSRFSGSGSGTXXTLTISSLQPEDFATYYCQQFSXSTWTFGQGTKLEIK

SEQ ID NO: 85 - protein, 119 aa, 人工序列(Artificial Sequence)
  UNSURE (46): Xaa is E or K
  UNSURE (63): Xaa is E or K
  UNSURE (72): Xaa is L or T
  UNSURE (77): Xaa is R or S
  UNSURE (97): Xaa is A or T
QVQLVQSGAEVKKPGASVKVSCKASGYTFTNYGMNWVRQAPGQGLXWMGWINTNTGEPTYAQXLQGRVTMTXDTSTXTAYMELRSLRSDDTAVYYCXRFSHLRGPMDYWGQGTLVTVSS

SEQ ID NO: 86 - protein, 112 aa, 人工序列(Artificial Sequence)
  UNSURE (2): Xaa is I or A
DXQMTQSPSSLSASVGDRVTITCRSSQSLVHSNGYTYLHWYQQKPGKAPKLLIYKVSNRFSGVPSRFSGSGSGTDFTLTISSLQPEDFATYYCSQSTHVPPTFGQGTKLEIK

SEQ ID NO: 87 - protein, 120 aa, 人工序列(Artificial Sequence)
  UNSURE (24): Xaa is A or V
  UNSURE (72): Xaa is R or G
  UNSURE (77): Xaa is S or N
  UNSURE (97): Xaa is A or T
QVQLVQSGAEVKKPGASVKVSCKXSGFNIEDDYIEWVRQAPGQGLEWMGRIDPANDKTKYAQKFQGRVTMTXDTSTXTVYMELSSLRSEDTAVYYCXRPGLRRYYSMDYWGQGTLVTVSS

SEQ ID NO: 88 - protein, 107 aa, 人工序列(Artificial Sequence)
  UNSURE (63): Xaa is S or I
  UNSURE (68): Xaa is S or G
DIQMTQSPSSLSASVGDRVTITCKASENVVSYVSWYQQKPGKAPKLLIYGASNRYTGVPSRFXGSGSXTDFTLTISSLQPEDFATYYCGQSYSYPLTFGQGTKLEIK

SEQ ID NO: 89 - protein, 443 aa, 人工序列(Artificial Sequence)
QVQLKESGPGLVAPSQSLSITCTVSGFSLTNYGVHWVRQPPGKGLEWLGIIWAGGSTNYNSALMSRLSISKDNSKSQVFLKMNSLQTDDTAMYYCARDDYASMDYWGQGTSVTVSSASTKGPSVFPLAPCSRSTSESTAALGCLVKDYFPEPVTVSWNSGALTSGVHTFPAVLQSSGLYSLSSVVTVPSSSLGTKTYTCNVDHKPSNTKVDKRVESKYGPPCPPCPAPEFLGGPSVFLFPPKPKDTLMISRTPEVTCVVVDVSQEDPEVQFNWYVDGVEVHNAKTKPREEQFNSTYRVVSVLTVLHQDWLNGKEYKCKVSNKGLPSSIEKTISKAKGQPREPQVYTLPPSQEEMTKNQVSLTCLVKGFYPSDIAVEWESNGQPENNYKTTPPVLDSDGSFFLYSRLTVDKSRWQEGNVFSCSVMHEALHNHYTQKSLSLSLGK

SEQ ID NO: 90 - DNA, 1332 bp, 人工序列(Artificial Sequence)
caggtgcagctgaaggagtctggaccaggactggtggctccatctcagtccctgagcatcacctgcacagtgtccggcttcagcctgaccaactacggagtgcactgggtgaggcagccacctggcaagggactggagtggctgggcatcatctgggctggcggctccacaaactataattctgccctgatgtcccggctgtctatctccaaggacaacagcaagtctcaggtgtttctgaagatgaatagcctgcagaccgacgatacagccatgtactattgtgctagggacgattacgccagcatggattattggggccagggcacctctgtgacagtgtccagcgcctctacaaagggcccttccgtgttcccactggctccctgctccagaagcacatctgagtccaccgccgctctgggctgtctggtgaaggactacttccctgagccagtgaccgtgtcctggaacagcggcgccctgacatctggcgtgcacacctttccagctgtgctgcagtccagcggcctgtactccctgtcttccgtggtgacagtgcccagctcttccctgggcaccaagacatatacctgcaacgtggaccataagccttccaataccaaggtggataagagggtggagagcaagtacggaccaccttgcccaccatgtccagctcctgagtttctgggaggaccatccgtgttcctgtttcctccaaagcctaaggacaccctgatgatcagccggacacctgaggtgacctgcgtggtggtggacgtgtctcaggaggatccagaggtgcagttcaactggtacgtggatggcgtggaggtgcacaatgctaagaccaagccaagagaggagcagtttaattccacataccgcgtggtgagcgtgctgaccgtgctgcatcaggattggctgaacggcaaggagtataagtgcaaggtgtccaataagggcctgcccagctctatcgagaagacaatcagcaaggctaagggacagcctagggagccacaggtgtacaccctgcccccttctcaggaggagatgacaaagaaccaggtgtccctgacctgtctggtgaagggcttctatccaagcgacatcgctgtggagtgggagtctaatggccagcccgagaacaattacaagaccacaccacccgtgctggactctgatggctccttctttctgtattctaggctgacagtggataagtcccggtggcaggagggcaacgtgtttagctgctctgtgatgcacgaggccctgcacaatcattatacccagaagtccctgagcctgtctctgggcaagtga

SEQ ID NO: 91 - protein, 219 aa, 人工序列(Artificial Sequence)
DAFMTQTPLSLPVSLGDQASISCRSSQSLVHSNGNTYLHWYLQKPGQSPKLLIYKVSNRFSGVPDRFSGSGSGTDFTLKISRVEAEDLGVYFCSQSTHVPYTLGGGTKLEIKRTVAAPSVFIFPPSDEQLKSGTASVVCLLNNFYPREAKVQWKVDNALQSGNSQESVTEQDSKDSTYSLSSTLTLSKADYEKHKVYACEVTHQGLSSPVTKSFNRGEC

SEQ ID NO: 92 - DNA, 660 bp, 人工序列(Artificial Sequence)
gacgccttcatgacccagacaccactgtccctgcctgtgagcctgggcgatcaggcttctatctcctgcagatccagccagtctctggtgcactccaacggcaatacatacctgcattggtatctgcagaagccaggccagtcccccaagctgctgatctacaaggtgagcaacaggttctctggcgtgcctgaccggtttagcggctctggctccggcaccgatttcacactgaagatctccagggtggaggctgaggacctgggcgtgtacttttgtagccagtctacccacgtgccatatacactgggcggcggcaccaagctggagatcaagcgtacggtggccgctcccagcgtgttcatctttcccccttctgacgagcagctgaagtctggcaccgcttccgtggtgtgcctgctgaacaatttctaccccagagaggccaaggtgcagtggaaggtggataacgctctgcagtccggcaatagccaggagtctgtgaccgagcaggactccaaggatagcacatattctctgtcttccaccctgacactgtctaaggccgactacgagaagcacaaggtgtatgcttgcgaggtgacccatcagggcctgagctctcctgtgacaaagtcctttaatcgcggcgagtgttga

SEQ ID NO: 93 - protein, 446 aa, 人工序列(Artificial Sequence)
EVQLQQSGPELKKPGETVKISCKASGYTFTNYGMNWVKQVPGKGLKWMGWINTNTGEPTYAEEFKGRFAFSLETSARTAFLQINNLKNEDTATYFCTRFSHLRGPMDYWGQGASVTVSSASTKGPSVFPLAPCSRSTSESTAALGCLVKDYFPEPVTVSWNSGALTSGVHTFPAVLQSSGLYSLSSVVTVPSSSLGTKTYTCNVDHKPSNTKVDKRVESKYGPPCPPCPAPEFLGGPSVFLFPPKPKDTLMISRTPEVTCVVVDVSQEDPEVQFNWYVDGVEVHNAKTKPREEQFNSTYRVVSVLTVLHQDWLNGKEYKCKVSNKGLPSSIEKTISKAKGQPREPQVYTLPPSQEEMTKNQVSLTCLVKGFYPSDIAVEWESNGQPENNYKTTPPVLDSDGSFFLYSRLTVDKSRWQEGNVFSCSVMHEALHNHYTQKSLSLSLGK

SEQ ID NO: 94 - DNA, 1341 bp, 人工序列(Artificial Sequence)
gaggtgcagctgcagcagtctggccccgagctgaagaagcctggcgagaccgtgaagatctcttgcaaggcctccggctacaccttcacaaactatggcatgaattgggtgaagcaggtgccaggcaagggcctgaagtggatgggctggatcaacaccaatacaggcgagcccacatacgccgaggagttcaagggcagattcgcttttagcctggagacctctgcccgcacagcttttctgcagatcaacaatctgaagaacgaggacaccgccacatacttctgtaccaggttttcccacctgcggggccccatggattattggggccagggcgctagcgtgacagtgtccagcgcctctacaaagggcccttccgtgttcccactggctccctgctccagaagcacatctgagtccaccgccgctctgggctgtctggtgaaggactacttccctgagccagtgaccgtgtcctggaacagcggcgccctgacatctggcgtgcacacctttccagctgtgctgcagtccagcggcctgtactccctgtcttccgtggtgacagtgcccagctcttccctgggcaccaagacatatacctgcaacgtggaccataagccttccaataccaaggtggataagagggtggagagcaagtacggaccaccttgcccaccatgtccagctcctgagtttctgggaggaccatccgtgttcctgtttcctccaaagcctaaggacaccctgatgatcagccggacacctgaggtgacctgcgtggtggtggacgtgtctcaggaggatccagaggtgcagttcaactggtacgtggatggcgtggaggtgcacaatgctaagaccaagccaagagaggagcagtttaattccacataccgcgtggtgagcgtgctgaccgtgctgcatcaggattggctgaacggcaaggagtataagtgcaaggtgtccaataagggcctgcccagctctatcgagaagacaatcagcaaggctaagggacagcctagggagccacaggtgtacaccctgcccccttctcaggaggagatgacaaagaaccaggtgtccctgacctgtctggtgaagggcttctatccaagcgacatcgctgtggagtgggagtctaatggccagcccgagaacaattacaagaccacaccacccgtgctggactctgatggctccttctttctgtattctaggctgacagtggataagtcccggtggcaggagggcaacgtgtttagctgctctgtgatgcacgaggccctgcacaatcattatacccagaagtccctgagcctgtctctgggcaagtga

SEQ ID NO: 95 - protein, 219 aa, 人工序列(Artificial Sequence)
DAVMTQTPLSLPVSLGDQASISCRSSQSLVHSNGYTYLHWYLQKPGQSPKLLIYKVSNRFSGVPDRFSGSGSGTDFTLKISRLEAEDLGVYFCSQSTHVPPTFGGGTKLEIKRTVAAPSVFIFPPSDEQLKSGTASVVCLLNNFYPREAKVQWKVDNALQSGNSQESVTEQDSKDSTYSLSSTLTLSKADYEKHKVYACEVTHQGLSSPVTKSFNRGEC

SEQ ID NO: 96 - DNA, 660 bp, 人工序列(Artificial Sequence)
gacgccgtgatgacccagacaccactgtccctgcccgtgagcctgggcgatcaggcttctatctcctgcagatccagccagtctctggtgcactccaacggctacacatatctgcattggtacctgcagaagcctggccagtccccaaagctgctgatctataaggtgagcaataggttctctggagtgccagaccggtttagcggatctggatccggcaccgatttcacactgaagatctccaggctggaggctgaggacctgggcgtgtacttctgtagccagtctacccacgtgccccctacatttggcggcggcaccaagctggagatcaagcgtacggtggccgctcccagcgtgttcatctttcccccttctgacgagcagctgaagtctggcaccgcttccgtggtgtgcctgctgaacaatttctaccccagagaggccaaggtgcagtggaaggtggataacgctctgcagtccggcaatagccaggagtctgtgaccgagcaggactccaaggatagcacatattctctgtcttccaccctgacactgtctaaggccgactacgagaagcacaaggtgtatgcttgcgaggtgacccatcagggcctgagctctcctgtgacaaagtcctttaatcgcggcgagtgttga

SEQ ID NO: 97 - protein, 439 aa, 人工序列(Artificial Sequence)
EVMLVESGGGLVQPGGSLKLSCAASGFTFSNYYMSWVRQTPEKRLEWVAYISSGGGSTYYPDSVKGRFTISRDNAKNTLYLQMSSLKSEDTAMYYCAWFAYWGQGTLVTVSAASTKGPSVFPLAPCSRSTSESTAALGCLVKDYFPEPVTVSWNSGALTSGVHTFPAVLQSSGLYSLSSVVTVPSSSLGTKTYTCNVDHKPSNTKVDKRVESKYGPPCPPCPAPEFLGGPSVFLFPPKPKDTLMISRTPEVTCVVVDVSQEDPEVQFNWYVDGVEVHNAKTKPREEQFNSTYRVVSVLTVLHQDWLNGKEYKCKVSNKGLPSSIEKTISKAKGQPREPQVYTLPPSQEEMTKNQVSLTCLVKGFYPSDIAVEWESNGQPENNYKTTPPVLDSDGSFFLYSRLTVDKSRWQEGNVFSCSVMHEALHNHYTQKSLSLSLGK

SEQ ID NO: 98 - DNA, 1320 bp, 人工序列(Artificial Sequence)
gaagtgatgctggtggagagcggaggaggactggtgcagccaggaggcagcctgaagctgtcttgcgccgcttccggcttcacctttagcaactactatatgtcttgggtgagacagacacccgagaagcgcctggagtgggtggcttacatctccagcggaggaggatccacctactatcctgacagcgtgaagggcaggttcaccatctctcgggataacgccaagaatacactgtacctgcagatgtcttccctgaagtccgaggacacagctatgtactattgtgcctggtttgcttattggggccagggcaccctggtgacagtgtctgctgcctctacaaagggcccttccgtgttcccactggctccctgctccagaagcacatctgagtccaccgccgctctgggctgtctggtgaaggactacttccctgagccagtgaccgtgtcctggaacagcggcgccctgacatctggcgtgcacacctttccagctgtgctgcagtccagcggcctgtactccctgtcttccgtggtgacagtgcccagctcttccctgggcaccaagacatatacctgcaacgtggaccataagccttccaataccaaggtggataagagggtggagagcaagtacggaccaccttgcccaccatgtccagctcctgagtttctgggaggaccatccgtgttcctgtttcctccaaagcctaaggacaccctgatgatcagccggacacctgaggtgacctgcgtggtggtggacgtgtctcaggaggatccagaggtgcagttcaactggtacgtggatggcgtggaggtgcacaatgctaagaccaagccaagagaggagcagtttaattccacataccgcgtggtgagcgtgctgaccgtgctgcatcaggattggctgaacggcaaggagtataagtgcaaggtgtccaataagggcctgcccagctctatcgagaagacaatcagcaaggctaagggacagcctagggagccacaggtgtacaccctgcccccttctcaggaggagatgacaaagaaccaggtgtccctgacctgtctggtgaagggcttctatccaagcgacatcgctgtggagtgggagtctaatggccagcccgagaacaattacaagaccacaccacccgtgctggactctgatggctccttctttctgtattctaggctgacagtggataagtcccggtggcaggagggcaacgtgtttagctgctctgtgatgcacgaggccctgcacaatcattatacccagaagtccctgagcctgtctctgggcaagtga

SEQ ID NO: 99 - protein, 219 aa, 人工序列(Artificial Sequence)
DAVVTQTPLTLSVTIGQPASISCKSSQSLLDSDGKTYLNWLLQRPGQSPKRLIYLVSKLDSGVPDRFTGSGSGTDFTLKISRVEAEDLGVYYCWQGTHFPLTFGAGTKLELKRTVAAPSVFIFPPSDEQLKSGTASVVCLLNNFYPREAKVQWKVDNALQSGNSQESVTEQDSKDSTYSLSSTLTLSKADYEKHKVYACEVTHQGLSSPVTKSFNRGEC

SEQ ID NO: 100 - DNA, 660 bp, 人工序列(Artificial Sequence)
gacgccgtggtgacccagacaccactgaccctgtccgtgacaatcggccagcccgcttctatctcctgcaagtccagccagtccctgctggacagcgatggcaagacatacctgaactggctgctgcagaggccaggacagagccctaagcggctgatctatctggtgtctaagctggactccggcgtgcctgatagattcaccggcagcggctctggcaccgactttacactgaagatctctcgcgtggaggccgaggatctgggcgtgtactattgttggcagggcacccacttcccactgacatttggcgctggcaccaagctggagctgaagcgtacggtggccgctcccagcgtgttcatctttcccccttctgacgagcagctgaagtctggcaccgcttccgtggtgtgcctgctgaacaatttctaccccagagaggccaaggtgcagtggaaggtggataacgctctgcagtccggcaatagccaggagtctgtgaccgagcaggactccaaggatagcacatattctctgtcttccaccctgacactgtctaaggccgactacgagaagcacaaggtgtatgcttgcgaggtgacccatcagggcctgagctctcctgtgacaaagtcctttaatcgcggcgagtgttga

SEQ ID NO: 101 - protein, 444 aa, 人工序列(Artificial Sequence)
EVQLQQSVAELMKPGASVKIYCKATGYTFSRYWIEWVKQRPGHGLEWIGEFIPGSDTTNFNEKFKGKATFTAEISSNTAYMQLSSLTSEDSAVYFCARGGLRRMDYWGQGTSVTVSSASTKGPSVFPLAPCSRSTSESTAALGCLVKDYFPEPVTVSWNSGALTSGVHTFPAVLQSSGLYSLSSVVTVPSSSLGTKTYTCNVDHKPSNTKVDKRVESKYGPPCPPCPAPEFLGGPSVFLFPPKPKDTLMISRTPEVTCVVVDVSQEDPEVQFNWYVDGVEVHNAKTKPREEQFNSTYRVVSVLTVLHQDWLNGKEYKCKVSNKGLPSSIEKTISKAKGQPREPQVYTLPPSQEEMTKNQVSLTCLVKGFYPSDIAVEWESNGQPENNYKTTPPVLDSDGSFFLYSRLTVDKSRWQEGNVFSCSVMHEALHNHYTQKSLSLSLGK

SEQ ID NO: 102 - DNA, 1335 bp, 人工序列(Artificial Sequence)
gaggtgcagctgcagcagtctgtggccgagctgatgaagccaggcgcttccgtgaagatctactgcaaggccaccggctacacattcagcagatattggatcgagtgggtgaagcagaggccaggacacggactggagtggatcggcgagttcatccctggctctgacaccacaaacttcaatgagaagtttaagggcaaggccacctttacagctgagatctccagcaacaccgcttatatgcagctgtcttccctgacatccgaggacagcgccgtgtacttttgtgctaggggcggcctgaggcggatggattattggggccagggcacctccgtgacagtgagctctgcctctacaaagggcccttccgtgttcccactggctccctgctccagaagcacatctgagtccaccgccgctctgggctgtctggtgaaggactacttccctgagccagtgaccgtgtcctggaacagcggcgccctgacatctggcgtgcacacctttccagctgtgctgcagtccagcggcctgtactccctgtcttccgtggtgacagtgcccagctcttccctgggcaccaagacatatacctgcaacgtggaccataagccttccaataccaaggtggataagagggtggagagcaagtacggaccaccttgcccaccatgtccagctcctgagtttctgggaggaccatccgtgttcctgtttcctccaaagcctaaggacaccctgatgatcagccggacacctgaggtgacctgcgtggtggtggacgtgtctcaggaggatccagaggtgcagttcaactggtacgtggatggcgtggaggtgcacaatgctaagaccaagccaagagaggagcagtttaattccacataccgcgtggtgagcgtgctgaccgtgctgcatcaggattggctgaacggcaaggagtataagtgcaaggtgtccaataagggcctgcccagctctatcgagaagacaatcagcaaggctaagggacagcctagggagccacaggtgtacaccctgcccccttctcaggaggagatgacaaagaaccaggtgtccctgacctgtctggtgaagggcttctatccaagcgacatcgctgtggagtgggagtctaatggccagcccgagaacaattacaagaccacaccacccgtgctggactctgatggctccttctttctgtattctaggctgacagtggataagtcccggtggcaggagggcaacgtgtttagctgctctgtgatgcacgaggccctgcacaatcattatacccagaagtccctgagcctgtctctgggcaagtga

SEQ ID NO: 103 - protein, 215 aa, 人工序列(Artificial Sequence)
DIVMTQTPAIMSASPGEKVTMTCRASSSVSSTYLHWYQQKSGASPKLWIYTTSTLASGVPARFSGSGSGTSYSLTISSVEAEDAATYYCQQFSDSTWTFGGGTKLEIKRTVAAPSVFIFPPSDEQLKSGTASVVCLLNNFYPREAKVQWKVDNALQSGNSQESVTEQDSKDSTYSLSSTLTLSKADYEKHKVYACEVTHQGLSSPVTKSFNRGEC

SEQ ID NO: 104 - DNA, 648 bp, 人工序列(Artificial Sequence)
gacatcgtgatgacccagacacccgccatcatgtccgcctctcctggcgagaaggtgaccatgacatgcagggcctccagctccgtgtccagcacctacctgcactggtatcagcagaagagcggcgcttctccaaagctgtggatctacaccacatccacactggctagcggagtgccagctcggttctccggaagcggatctggcacctcctatagcctgacaatctcttccgtggaggccgaggacgccgctacctactattgtcagcagttctctgattccacctggacatttggcggcggcacaaagctggagatcaagcgtacggtggccgctcccagcgtgttcatctttcccccttctgacgagcagctgaagtctggcaccgcttccgtggtgtgcctgctgaacaatttctaccccagagaggccaaggtgcagtggaaggtggataacgctctgcagtccggcaatagccaggagtctgtgaccgagcaggactccaaggatagcacatattctctgtcttccaccctgacactgtctaaggccgactacgagaagcacaaggtgtatgcttgcgaggtgacccatcagggcctgagctctcctgtgacaaagtcctttaatcgcggcgagtgttga

SEQ ID NO: 105 - protein, 447 aa, 人工序列(Artificial Sequence)
EVQLQQSGAEVARPGASVKLSCTVSGFNIEDDYIEWVKQRPEQGLEWIGRIDPANDKTKYAPKFQDKATITGDTSSNTAYLQLSSLTSEDTAVYYCTRPGLRRYYSMDYWGQGTSVTVSSASTKGPSVFPLAPCSRSTSESTAALGCLVKDYFPEPVTVSWNSGALTSGVHTFPAVLQSSGLYSLSSVVTVPSSSLGTKTYTCNVDHKPSNTKVDKRVESKYGPPCPPCPAPEFLGGPSVFLFPPKPKDTLMISRTPEVTCVVVDVSQEDPEVQFNWYVDGVEVHNAKTKPREEQFNSTYRVVSVLTVLHQDWLNGKEYKCKVSNKGLPSSIEKTISKAKGQPREPQVYTLPPSQEEMTKNQVSLTCLVKGFYPSDIAVEWESNGQPENNYKTTPPVLDSDGSFFLYSRLTVDKSRWQEGNVFSCSVMHEALHNHYTQKSLSLSLGK

SEQ ID NO: 106 - DNA, 1344 bp, 人工序列(Artificial Sequence)
gaggtgcagctgcagcagtctggagctgaggtggctaggccaggagcttccgtgaagctgagctgcaccgtgtctggcttcaacatcgaggacgattacatcgagtgggtgaagcagagaccagagcagggactggagtggatcggaaggatcgaccccgccaacgataagacaaagtacgctcctaagtttcaggacaaggccaccatcacaggcgatacctccagcaatacagcttatctgcagctgtcttccctgacctccgaggacacagccgtgtactattgtaccagacccggcctgaggcggtactattccatggattattggggccagggcaccagcgtgacagtgagctctgcctctacaaagggcccttccgtgttcccactggctccctgctccagaagcacatctgagtccaccgccgctctgggctgtctggtgaaggactacttccctgagccagtgaccgtgtcctggaacagcggcgccctgacatctggcgtgcacacctttccagctgtgctgcagtccagcggcctgtactccctgtcttccgtggtgacagtgcccagctcttccctgggcaccaagacatatacctgcaacgtggaccataagccttccaataccaaggtggataagagggtggagagcaagtacggaccaccttgcccaccatgtccagctcctgagtttctgggaggaccatccgtgttcctgtttcctccaaagcctaaggacaccctgatgatcagccggacacctgaggtgacctgcgtggtggtggacgtgtctcaggaggatccagaggtgcagttcaactggtacgtggatggcgtggaggtgcacaatgctaagaccaagccaagagaggagcagtttaattccacataccgcgtggtgagcgtgctgaccgtgctgcatcaggattggctgaacggcaaggagtataagtgcaaggtgtccaataagggcctgcccagctctatcgagaagacaatcagcaaggctaagggacagcctagggagccacaggtgtacaccctgcccccttctcaggaggagatgacaaagaaccaggtgtccctgacctgtctggtgaagggcttctatccaagcgacatcgctgtggagtgggagtctaatggccagcccgagaacaattacaagaccacaccacccgtgctggactctgatggctccttctttctgtattctaggctgacagtggataagtcccggtggcaggagggcaacgtgtttagctgctctgtgatgcacgaggccctgcacaatcattatacccagaagtccctgagcctgtctctgggcaagtga

SEQ ID NO: 107 - protein, 214 aa, 人工序列(Artificial Sequence)
NIVLTQSPKSMSMSVGERVTLSCKASENVVSYVSWYQQKPEQSPKLLIYGASNRYTGVPDRFIGSGSSTDFTLIISSFQPEDLADYHCGQSYSYPLTFGAGTKLELKRTVAAPSVFIFPPSDEQLKSGTASVVCLLNNFYPREAKVQWKVDNALQSGNSQESVTEQDSKDSTYSLSSTLTLSKADYEKHKVYACEVTHQGLSSPVTKSFNRGEC

SEQ ID NO: 108 - DNA, 645 bp, 人工序列(Artificial Sequence)
aacatcgtgctgacccagtcccctaagagcatgtctatgtccgtgggcgagagggtgacactgtcttgcaaggcctccgagaacgtggtgtcctacgtgagctggtatcagcagaagcccgagcagagccctaagctgctgatctacggcgcttctaataggtataccggagtgccagaccggttcatcggatccggctccagcaccgatttcacactgatcatctcttcctttcagccagaggacctggccgattaccactgtggccagagctactcttatcccctgacctttggcgctggcacaaagctggagctgaagcgtacggtggccgctcccagcgtgttcatctttcccccttctgacgagcagctgaagtctggcaccgcttccgtggtgtgcctgctgaacaatttctaccccagagaggccaaggtgcagtggaaggtggataacgctctgcagtccggcaatagccaggagtctgtgaccgagcaggactccaaggatagcacatattctctgtcttccaccctgacactgtctaaggccgactacgagaagcacaaggtgtatgcttgcgaggtgacccatcagggcctgagctctcctgtgacaaagtcctttaatcgcggcgagtgttga

SEQ ID NO: 109 - protein, 444 aa, 人工序列(Artificial Sequence)
QVQLVQSGAEVKKPGSSVKVSCKASGYTFSRYWIEWVRQAPGQGLEWMGEFIPGSDTTNYAQKFQGRVTITADISTSTAYMELSSLRSEDTAVYYCARGGLRRMDYWGQGTLVTVSSASTKGPSVFPLAPCSRSTSESTAALGCLVKDYFPEPVTVSWNSGALTSGVHTFPAVLQSSGLYSLSSVVTVPSSSLGTKTYTCNVDHKPSNTKVDKRVESKYGPPCPPCPAPEFLGGPSVFLFPPKPKDTLMISRTPEVTCVVVDVSQEDPEVQFNWYVDGVEVHNAKTKPREEQFNSTYRVVSVLTVLHQDWLNGKEYKCKVSNKGLPSSIEKTISKAKGQPREPQVYTLPPSQEEMTKNQVSLTCLVKGFYPSDIAVEWESNGQPENNYKTTPPVLDSDGSFFLYSRLTVDKSRWQEGNVFSCSVMHEALHNHYTQKSLSLSLGK

SEQ ID NO: 110 - DNA, 1335 bp, 人工序列(Artificial Sequence)
caggtgcagctggtgcagagcggagctgaggtgaagaagccaggctccagcgtgaaggtgtcttgcaaggcttccggctacaccttctctagatattggatcgagtgggtgcgccaggctccaggacagggactggagtggatgggcgagttcatccctggctccgacaccacaaactacgctcagaagtttcagggcagggtgaccatcacagccgatatctccaccagcacagcttatatggagctgtcttccctgaggagcgaggacacagccgtgtactattgtgctagaggcggcctgaggcggatggattactggggccagggcaccctggtgacagtgagctctgcctctacaaagggcccttccgtgttcccactggctccctgctccagaagcacatctgagtccaccgccgctctgggctgtctggtgaaggactacttccctgagccagtgaccgtgtcctggaacagcggcgccctgacatctggcgtgcacacctttccagctgtgctgcagtccagcggcctgtactccctgtcttccgtggtgacagtgcccagctcttccctgggcaccaagacatatacctgcaacgtggaccataagccttccaataccaaggtggataagagggtggagagcaagtacggaccaccttgcccaccatgtccagctcctgagtttctgggaggaccatccgtgttcctgtttcctccaaagcctaaggacaccctgatgatcagccggacacctgaggtgacctgcgtggtggtggacgtgtctcaggaggatccagaggtgcagttcaactggtacgtggatggcgtggaggtgcacaatgctaagaccaagccaagagaggagcagtttaattccacataccgcgtggtgagcgtgctgaccgtgctgcatcaggattggctgaacggcaaggagtataagtgcaaggtgtccaataagggcctgcccagctctatcgagaagacaatcagcaaggctaagggacagcctagggagccacaggtgtacaccctgcccccttctcaggaggagatgacaaagaaccaggtgtccctgacctgtctggtgaagggcttctatccaagcgacatcgctgtggagtgggagtctaatggccagcccgagaacaattacaagaccacaccacccgtgctggactctgatggctccttctttctgtattctaggctgacagtggataagtcccggtggcaggagggcaacgtgtttagctgctctgtgatgcacgaggccctgcacaatcattatacccagaagtccctgagcctgtctctgggcaagtga

SEQ ID NO: 111 - protein, 215 aa, 人工序列(Artificial Sequence)
DIQMTQSPSSLSASVGDRVTITCRASSSVSSTYLHWYQQKPGKAPKLLIYTTSTLASGVPSRFSGSGSGTDFTLTISSLQPEDFATYYCQQFSDSTWTFGQGTKLEIKRTVAAPSVFIFPPSDEQLKSGTASVVCLLNNFYPREAKVQWKVDNALQSGNSQESVTEQDSKDSTYSLSSTLTLSKADYEKHKVYACEVTHQGLSSPVTKSFNRGEC

SEQ ID NO: 112 - DNA, 648 bp, 人工序列(Artificial Sequence)
gacatccagatgacacagagcccatccagcctgtccgccagcgtgggcgatagggtgaccatcacatgccgggcttcttccagcgtgtcttccacctacctgcactggtatcagcagaagcccggcaaggcccctaagctgctgatctacaccacaagcaccctggcttctggcgtgccatccaggttctctggctccggcagcggcacagactttaccctgacaatcagctctctgcagcccgaggacttcgccacctactattgtcagcagttctctgattccacctggacatttggccagggcacaaagctggagatcaagcgtacggtggccgctcccagcgtgttcatctttcccccttctgacgagcagctgaagtctggcaccgcttccgtggtgtgcctgctgaacaatttctaccccagagaggccaaggtgcagtggaaggtggataacgctctgcagtccggcaatagccaggagtctgtgaccgagcaggactccaaggatagcacatattctctgtcttccaccctgacactgtctaaggccgactacgagaagcacaaggtgtatgcttgcgaggtgacccatcagggcctgagctctcctgtgacaaagtcctttaatcgcggcgagtgttga

SEQ ID NO: 113 - protein, 444 aa, 人工序列(Artificial Sequence); identical to SEQ ID NO: 109

SEQ ID NO: 114 - DNA, 1335 bp, 人工序列(Artificial Sequence); identical to SEQ ID NO: 110

SEQ ID NO: 115 - protein, 215 aa, 人工序列(Artificial Sequence)
DIQMTQSPSSLSASVGDRVTITCRASSSVSSTYLHWYQQKPGKAPKLLIYTTSTLASGVPSRFSGSGSGTDFTLTISSLQPEDFATYYCQQFSESTWTFGQGTKLEIKRTVAAPSVFIFPPSDEQLKSGTASVVCLLNNFYPREAKVQWKVDNALQSGNSQESVTEQDSKDSTYSLSSTLTLSKADYEKHKVYACEVTHQGLSSPVTKSFNRGEC

SEQ ID NO: 116 - DNA, 648 bp, 人工序列(Artificial Sequence)
gacatccagatgacacagagcccatccagcctgtccgccagcgtgggcgatagggtgaccatcacatgccgggcttcttccagcgtgtcttccacctacctgcactggtatcagcagaagcccggcaaggcccctaagctgctgatctacaccacaagcaccctggcttctggcgtgccatccaggttctctggctccggcagcggcacagactttaccctgacaatcagctctctgcagcccgaggatttcgccacctactattgtcagcagttctctgagtccacctggacatttggccagggcacaaagctggagatcaagcgtacggtggccgctcccagcgtgttcatctttcccccttctgacgagcagctgaagtctggcaccgcttccgtggtgtgcctgctgaacaatttctaccccagagaggccaaggtgcagtggaaggtggataacgctctgcagtccggcaatagccaggagtctgtgaccgagcaggactccaaggatagcacatattctctgtcttccaccctgacactgtctaaggccgactacgagaagcacaaggtgtatgcttgcgaggtgacccatcagggcctgagctctcctgtgacaaagtcctttaatcgcggcgagtgttga

SEQ ID NO: 117 - protein, 444 aa, 人工序列(Artificial Sequence); identical to SEQ ID NO: 109

SEQ ID NO: 118 - DNA, 1335 bp, 人工序列(Artificial Sequence); identical to SEQ ID NO: 110

SEQ ID NO: 119 - protein, 215 aa, 人工序列(Artificial Sequence)
DIQMTQSPSSLSASVGDRVTITCRASSSVSSTYLHWYQQKPGKAPKLLIYTTSTLASGVPSRFSGSGSGTSYTLTISSLQPEDFATYYCQQFSDSTWTFGQGTKLEIKRTVAAPSVFIFPPSDEQLKSGTASVVCLLNNFYPREAKVQWKVDNALQSGNSQESVTEQDSKDSTYSLSSTLTLSKADYEKHKVYACEVTHQGLSSPVTKSFNRGEC

SEQ ID NO: 120 - DNA, 648 bp, 人工序列(Artificial Sequence)
gacatccagatgacacagagcccatccagcctgtccgccagcgtgggcgatagggtgaccatcacatgccgggcttcttccagcgtgtcttccacctacctgcactggtatcagcagaagcccggcaaggcccctaagctgctgatctacaccacaagcaccctggcttctggcgtgccatccaggttctctggctccggcagcggcacatcttataccctgacaatcagctctctgcagcccgaggactttgccacctactattgtcagcagttctctgattccacctggacatttggccagggcacaaagctggagatcaagcgtacggtggccgctcccagcgtgttcatctttcccccttctgacgagcagctgaagtctggcaccgcttccgtggtgtgcctgctgaacaatttctaccccagagaggccaaggtgcagtggaaggtggataacgctctgcagtccggcaatagccaggagtctgtgaccgagcaggactccaaggatagcacatattctctgtcttccaccctgacactgtctaaggccgactacgagaagcacaaggtgtatgcttgcgaggtgacccatcagggcctgagctctcctgtgacaaagtcctttaatcgcggcgagtgttga

SEQ ID NO: 121 - protein, 444 aa, 人工序列(Artificial Sequence); identical to SEQ ID NO: 109

SEQ ID NO: 122 - DNA, 1335 bp, 人工序列(Artificial Sequence); identical to SEQ ID NO: 110

SEQ ID NO: 123 - protein, 215 aa, 人工序列(Artificial Sequence)
DIQMTQSPSSLSASVGDRVTITCRASSSVSSTYLHWYQQKPGKAPKLLIYTTSTLASGVPSRFSGSGSGTSYTLTISSLQPEDFATYYCQQFSESTWTFGQGTKLEIKRTVAAPSVFIFPPSDEQLKSGTASVVCLLNNFYPREAKVQWKVDNALQSGNSQESVTEQDSKDSTYSLSSTLTLSKADYEKHKVYACEVTHQGLSSPVTKSFNRGEC

SEQ ID NO: 124 - DNA, 648 bp, 人工序列(Artificial Sequence)
gacatccagatgacacagagcccatccagcctgtccgccagcgtgggcgatagggtgaccatcacatgccgggcttcttccagcgtgtcttccacctacctgcactggtatcagcagaagcccggcaaggcccctaagctgctgatctacaccacaagcaccctggcttctggcgtgccatccaggttctctggctccggcagcggcacatcttataccctgacaatcagctctctgcagcccgaggactttgccacctactattgtcagcagttctctgagtccacctggacatttggccagggcacaaagctggagatcaagcgtacggtggccgctcccagcgtgttcatctttcccccttctgacgagcagctgaagtctggcaccgcttccgtggtgtgcctgctgaacaatttctaccccagagaggccaaggtgcagtggaaggtggataacgctctgcagtccggcaatagccaggagtctgtgaccgagcaggactccaaggatagcacatattctctgtcttccaccctgacactgtctaaggccgactacgagaagcacaaggtgtatgcttgcgaggtgacccatcagggcctgagctctcctgtgacaaagtcctttaatcgcggcgagtgttga

SEQ ID NO: 125 - protein, 444 aa, 人工序列(Artificial Sequence); identical to SEQ ID NO: 109

SEQ ID NO: 126 - DNA, 1335 bp, 人工序列(Artificial Sequence); identical to SEQ ID NO: 110

SEQ ID NO: 127 - protein, 215 aa, 人工序列(Artificial Sequence)
DIQMTQSPSSLSASVGDRVTITCRASSSVSSTYLHWYQQKPGKAPKLWIYTTSTLASGVPSRFSGSGSGTSYTLTISSLQPEDFATYYCQQFSDSTWTFGQGTKLEIKRTVAAPSVFIFPPSDEQLKSGTASVVCLLNNFYPREAKVQWKVDNALQSGNSQESVTEQDSKDSTYSLSSTLTLSKADYEKHKVYACEVTHQGLSSPVTKSFNRGEC

SEQ ID NO: 128 - DNA, 648 bp, 人工序列(Artificial Sequence)
gacatccagatgacacagagcccatccagcctgtccgccagcgtgggcgatagggtgaccatcacatgccgggcttcttccagcgtgtcttccacctacctgcactggtatcagcagaagcccggcaaggcccctaagctgtggatctacaccacaagcaccctggcttctggcgtgccatccaggttctctggctccggcagcggcacatcttataccctgacaatcagctctctgcagcccgaggactttgccacctactattgtcagcagttctctgattccacctggacatttggccagggcacaaagctggagatcaagcgtacggtggccgctcccagcgtgttcatctttcccccttctgacgagcagctgaagtctggcaccgcttccgtggtgtgcctgctgaacaatttctaccccagagaggccaaggtgcagtggaaggtggataacgctctgcagtccggcaatagccaggagtctgtgaccgagcaggactccaaggatagcacatattctctgtcttccaccctgacactgtctaaggccgactacgagaagcacaaggtgtatgcttgcgaggtgacccatcagggcctgagctctcctgtgacaaagtcctttaatcgcggcgagtgttga

SEQ ID NO: 129 - protein, 444 aa, 人工序列(Artificial Sequence); identical to SEQ ID NO: 109

SEQ ID NO: 130 - DNA, 1335 bp, 人工序列(Artificial Sequence); identical to SEQ ID NO: 110

SEQ ID NO: 131 - protein, 215 aa, 人工序列(Artificial Sequence)
DIQMTQSPSSLSASVGDRVTITCRASSSVSSTYLHWYQQKPGKAPKLWIYTTSTLASGVPSRFSGSGSGTSYTLTISSLQPEDFATYYCQQFSESTWTFGQGTKLEIKRTVAAPSVFIFPPSDEQLKSGTASVVCLLNNFYPREAKVQWKVDNALQSGNSQESVTEQDSKDSTYSLSSTLTLSKADYEKHKVYACEVTHQGLSSPVTKSFNRGEC

SEQ ID NO: 132 - DNA, 648 bp, 人工序列(Artificial Sequence)
gacatccagatgacacagagcccatccagcctgtccgccagcgtgggcgatagggtgaccatcacatgccgggcttcttccagcgtgtcttccacctacctgcactggtatcagcagaagcccggcaaggcccctaagctgtggatctacaccacaagcaccctggcttctggcgtgccatccaggttctctggctccggcagcggcacatcttataccctgacaatcagctctctgcagcccgaggactttgccacctactattgtcagcagttctctgagtccacctggacatttggccagggcacaaagctggagatcaagcgtacggtggccgctcccagcgtgttcatctttcccccttctgacgagcagctgaagtctggcaccgcttccgtggtgtgcctgctgaacaatttctaccccagagaggccaaggtgcagtggaaggtggataacgctctgcagtccggcaatagccaggagtctgtgaccgagcaggactccaaggatagcacatattctctgtcttccaccctgacactgtctaaggccgactacgagaagcacaaggtgtatgcttgcgaggtgacccatcagggcctgagctctcctgtgacaaagtcctttaatcgcggcgagtgttga

SEQ ID NO: 133 - protein, 444 aa, 人工序列(Artificial Sequence)
QVQLVQSGAEVKKPGSSVKVSCKASGYTFSRYWIEWVRQAPGQGLEWMGEFIPGSDTTNYAQKFQGRVTITAEISTNTAYMELSSLRSEDTAVYYCARGGLRRMDYWGQGTLVTVSSASTKGPSVFPLAPCSRSTSESTAALGCLVKDYFPEPVTVSWNSGALTSGVHTFPAVLQSSGLYSLSSVVTVPSSSLGTKTYTCNVDHKPSNTKVDKRVESKYGPPCPPCPAPEFLGGPSVFLFPPKPKDTLMISRTPEVTCVVVDVSQEDPEVQFNWYVDGVEVHNAKTKPREEQFNSTYRVVSVLTVLHQDWLNGKEYKCKVSNKGLPSSIEKTISKAKGQPREPQVYTLPPSQEEMTKNQVSLTCLVKGFYPSDIAVEWESNGQPENNYKTTPPVLDSDGSFFLYSRLTVDKSRWQEGNVFSCSVMHEALHNHYTQKSLSLSLGK

SEQ ID NO: 134 - DNA, 1335 bp, 人工序列(Artificial Sequence)
caggtgcagctggtgcagagcggagctgaggtgaagaagccaggctccagcgtgaaggtgtcctgcaaggctagcggctacaccttctctagatattggatcgagtgggtgcgccaggctccaggacagggactggagtggatgggcgagttcatccctggctccgacaccacaaactacgctcagaagtttcagggcagggtgaccatcacagccgagatctctaccaatacagcttatatggagctgtcttccctgaggtccgaggacacagccgtgtactattgtgctagaggcggcctgaggcggatggattactggggccagggcaccctggtgacagtgagctctgcctctacaaagggcccttccgtgttcccactggctccctgctccagaagcacatctgagtccaccgccgctctgggctgtctggtgaaggactacttccctgagccagtgaccgtgtcctggaacagcggcgccctgacatctggcgtgcacacctttccagctgtgctgcagtccagcggcctgtactccctgtcttccgtggtgacagtgcccagctcttccctgggcaccaagacatatacctgcaacgtggaccataagccttccaataccaaggtggataagagggtggagagcaagtacggaccaccttgcccaccatgtccagctcctgagtttctgggaggaccatccgtgttcctgtttcctccaaagcctaaggacaccctgatgatcagccggacacctgaggtgacctgcgtggtggtggacgtgtctcaggaggatccagaggtgcagttcaactggtacgtggatggcgtggaggtgcacaatgctaagaccaagccaagagaggagcagtttaattccacataccgcgtggtgagcgtgctgaccgtgctgcatcaggattggctgaacggcaaggagtataagtgcaaggtgtccaataagggcctgcccagctctatcgagaagacaatcagcaaggctaagggacagcctagggagccacaggtgtacaccctgcccccttctcaggaggagatgacaaagaaccaggtgtccctgacctgtctggtgaagggcttctatccaagcgacatcgctgtggagtgggagtctaatggccagcccgagaacaattacaagaccacaccacccgtgctggactctgatggctccttctttctgtattctaggctgacagtggataagtcccggtggcaggagggcaacgtgtttagctgctctgtgatgcacgaggccctgcacaatcattatacccagaagtccctgagcctgtctctgggcaagtga

SEQ ID NO: 135 - protein, 215 aa, 人工序列(Artificial Sequence); identical to SEQ ID NO: 111

SEQ ID NO: 136 - DNA, 648 bp, 人工序列(Artificial Sequence); identical to SEQ ID NO: 112

SEQ ID NO: 137 - protein, 444 aa, 人工序列(Artificial Sequence); identical to SEQ ID NO: 133

SEQ ID NO: 138 - DNA, 1335 bp, 人工序列(Artificial Sequence); identical to SEQ ID NO: 134

SEQ ID NO: 139 - protein, 215 aa, 人工序列(Artificial Sequence); identical to SEQ ID NO: 115

SEQ ID NO: 140 - DNA, 648 bp, 人工序列(Artificial Sequence); identical to SEQ ID NO: 116

SEQ ID NO: 141 - protein, 444 aa, 人工序列(Artificial Sequence); identical to SEQ ID NO: 133

SEQ ID NO: 142 - DNA, 1335 bp, 人工序列(Artificial Sequence); identical to SEQ ID NO: 134

SEQ ID NO: 143 - protein, 215 aa, 人工序列(Artificial Sequence); identical to SEQ ID NO: 119

SEQ ID NO: 144 - DNA, 648 bp, 人工序列(Artificial Sequence); identical to SEQ ID NO: 120

SEQ ID NO: 145 - protein, 444 aa, 人工序列(Artificial Sequence); identical to SEQ ID NO: 133

SEQ ID NO: 146 - DNA, 1335 bp, 人工序列(Artificial Sequence); identical to SEQ ID NO: 134

SEQ ID NO: 147 - protein, 215 aa, 人工序列(Artificial Sequence); identical to SEQ ID NO: 123

SEQ ID NO: 148 - DNA, 648 bp, 人工序列(Artificial Sequence); identical to SEQ ID NO: 124

SEQ ID NO: 149 - protein, 444 aa, 人工序列(Artificial Sequence); identical to SEQ ID NO: 133

SEQ ID NO: 150 - DNA, 1335 bp, 人工序列(Artificial Sequence); identical to SEQ ID NO: 134

SEQ ID NO: 151 - protein, 215 aa, 人工序列(Artificial Sequence); identical to SEQ ID NO: 127

SEQ ID NO: 152 - DNA, 648 bp, 人工序列(Artificial Sequence); identical to SEQ ID NO: 128

SEQ ID NO: 153 - protein, 444 aa, 人工序列(Artificial Sequence); identical to SEQ ID NO: 133

SEQ ID NO: 154 - DNA, 1335 bp, 人工序列(Artificial Sequence); identical to SEQ ID NO: 134

SEQ ID NO: 155 - protein, 215 aa, 人工序列(Artificial Sequence); identical to SEQ ID NO: 131

SEQ ID NO: 156 - DNA, 648 bp, 人工序列(Artificial Sequence); identical to SEQ ID NO: 132

SEQ ID NO: 157 - protein, 446 aa, 人工序列(Artificial Sequence)
QVQLVQSGAEVKKPGASVKVSCKASGYTFTNYGMNWVRQAPGQGLEWMGWINTNTGEPTYAQKLQGRVTMTLDTSTRTAYMELRSLRSDDTAVYYCARFSHLRGPMDYWGQGTLVTVSSASTKGPSVFPLAPCSRSTSESTAALGCLVKDYFPEPVTVSWNSGALTSGVHTFPAVLQSSGLYSLSSVVTVPSSSLGTKTYTCNVDHKPSNTKVDKRVESKYGPPCPPCPAPEFLGGPSVFLFPPKPKDTLMISRTPEVTCVVVDVSQEDPEVQFNWYVDGVEVHNAKTKPREEQFNSTYRVVSVLTVLHQDWLNGKEYKCKVSNKGLPSSIEKTISKAKGQPREPQVYTLPPSQEEMTKNQVSLTCLVKGFYPSDIAVEWESNGQPENNYKTTPPVLDSDGSFFLYSRLTVDKSRWQEGNVFSCSVMHEALHNHYTQKSLSLSLGK

SEQ ID NO: 158 - DNA, 1341 bp, 人工序列(Artificial Sequence)
caggtgcagctggtgcagtccggagctgaggtgaagaagccaggagctagcgtgaaggtgtcttgcaaggcctccggctacaccttcacaaactatggcatgaattgggtgaggcaggctccaggacagggactggagtggatgggctggatcaacaccaatacaggcgagcctacatacgcccagaagctgcagggcagggtgaccatgacactggacaccagcacaagaaccgcttatatggagctgaggtctctgcggtccgacgataccgccgtgtactattgtgctagattttctcacctgaggggaccaatggattactggggacagggcacactggtgaccgtgtccagcgcctctacaaagggcccttccgtgttcccactggctccctgctccagaagcacatctgagtccaccgccgctctgggctgtctggtgaaggactacttccctgagccagtgaccgtgtcctggaacagcggcgccctgacatctggcgtgcacacctttccagctgtgctgcagtccagcggcctgtactccctgtcttccgtggtgacagtgcccagctcttccctgggcaccaagacatatacctgcaacgtggaccataagccttccaataccaaggtggataagagggtggagagcaagtacggaccaccttgcccaccatgtccagctcctgagtttctgggaggaccatccgtgttcctgtttcctccaaagcctaaggacaccctgatgatcagccggacacctgaggtgacctgcgtggtggtggacgtgtctcaggaggatccagaggtgcagttcaactggtacgtggatggcgtggaggtgcacaatgctaagaccaagccaagagaggagcagtttaattccacataccgcgtggtgagcgtgctgaccgtgctgcatcaggattggctgaacggcaaggagtataagtgcaaggtgtccaataagggcctgcccagctctatcgagaagacaatcagcaaggctaagggacagcctagggagccacaggtgtacaccctgcccccttctcaggaggagatgacaaagaaccaggtgtccctgacctgtctggtgaagggcttctatccaagcgacatcgctgtggagtgggagtctaatggccagcccgagaacaattacaagaccacaccacccgtgctggactctgatggctccttctttctgtattctaggctgacagtggataagtcccggtggcaggagggcaacgtgtttagctgctctgtgatgcacgaggccctgcacaatcattatacccagaagtccctgagcctgtctctgggcaagtga

SEQ ID NO: 159 - protein, 219 aa, 人工序列(Artificial Sequence)
DIQMTQSPSSLSASVGDRVTITCRSSQSLVHSNGYTYLHWYQQKPGKAPKLLIYKVSNRFSGVPSRFSGSGSGTDFTLTISSLQPEDFATYYCSQSTHVPPTFGQGTKLEIKRTVAAPSVFIFPPSDEQLKSGTASVVCLLNNFYPREAKVQWKVDNALQSGNSQESVTEQDSKDSTYSLSSTLTLSKADYEKHKVYACEVTHQGLSSPVTKSFNRGEC

SEQ ID NO: 160 - DNA, 660 bp, 人工序列(Artificial Sequence)
gacatccagatgacacagtccccatccagcctgtccgccagcgtgggcgatagggtgaccatcacatgccggtcttcccagagcctggtgcactctaacggctacacctatctgcattggtaccagcagaagccaggcaaggctcccaagctgctgatctataaggtgtccaatagattcagcggcgtgccttctcgcttttctggctccggcagcggcacagacttcaccctgacaatcagctctctgcagccagaggattttgccacctactattgttctcagtccacccacgtgccccctacattcggccagggcaccaagctggagatcaagcgtacggtggccgctcccagcgtgttcatctttcccccttctgacgagcagctgaagtctggcaccgcttccgtggtgtgcctgctgaacaatttctaccccagagaggccaaggtgcagtggaaggtggataacgctctgcagtccggcaatagccaggagtctgtgaccgagcaggactccaaggatagcacatattctctgtcttccaccctgacactgtctaaggccgactacgagaagcacaaggtgtatgcttgcgaggtgacccatcagggcctgagctctcctgtgacaaagtcctttaatcgcggcgagtgttga

SEQ ID NO: 161 - protein, 446 aa, 人工序列(Artificial Sequence)
QVQLVQSGAEVKKPGASVKVSCKASGYTFTNYGMNWVRQAPGQGLKWMGWINTNTGEPTYAQELQGRVTMTLDTSTRTAYMELRSLRSDDTAVYYCTRFSHLRGPMDYWGQGTLVTVSSASTKGPSVFPLAPCSRSTSESTAALGCLVKDYFPEPVTVSWNSGALTSGVHTFPAVLQSSGLYSLSSVVTVPSSSLGTKTYTCNVDHKPSNTKVDKRVESKYGPPCPPCPAPEFLGGPSVFLFPPKPKDTLMISRTPEVTCVVVDVSQEDPEVQFNWYVDGVEVHNAKTKPREEQFNSTYRVVSVLTVLHQDWLNGKEYKCKVSNKGLPSSIEKTISKAKGQPREPQVYTLPPSQEEMTKNQVSLTCLVKGFYPSDIAVEWESNGQPENNYKTTPPVLDSDGSFFLYSRLTVDKSRWQEGNVFSCSVMHEALHNHYTQKSLSLSLGK

SEQ ID NO: 162 - DNA, 1341 bp, 人工序列(Artificial Sequence)
caggtgcagctggtgcagtccggagctgaggtgaagaagccaggagctagcgtgaaggtgtcttgcaaggcctccggctacaccttcacaaactatggcatgaattgggtgaggcaggctccaggacagggcctgaagtggatgggatggatcaacaccaatacaggcgagcctacatacgcccaggagctgcagggcagggtgaccatgacactggacaccagcacaagaaccgcctatatggagctgaggtctctgcggtccgacgatacagccgtgtactattgtaccagattttctcacctgaggggaccaatggattactggggacagggcacactggtgaccgtgtccagcgcctctacaaagggcccttccgtgttcccactggctccctgctccagaagcacatctgagtccaccgccgctctgggctgtctggtgaaggactacttccctgagccagtgaccgtgtcctggaacagcggcgccctgacatctggcgtgcacacctttccagctgtgctgcagtccagcggcctgtactccctgtcttccgtggtgacagtgcccagctcttccctgggcaccaagacatatacctgcaacgtggaccataagccttccaataccaaggtggataagagggtggagagcaagtacggaccaccttgcccaccatgtccagctcctgagtttctgggaggaccatccgtgttcctgtttcctccaaagcctaaggacaccctgatgatcagccggacacctgaggtgacctgcgtggtggtggacgtgtctcaggaggatccagaggtgcagttcaactggtacgtggatggcgtggaggtgcacaatgctaagaccaagccaagagaggagcagtttaattccacataccgcgtggtgagcgtgctgaccgtgctgcatcaggattggctgaacggcaaggagtataagtgcaaggtgtccaataagggcctgcccagctctatcgagaagacaatcagcaaggctaagggacagcctagggagccacaggtgtacaccctgcccccttctcaggaggagatgacaaagaaccaggtgtccctgacctgtctggtgaagggcttctatccaagcgacatcgctgtggagtgggagtctaatggccagcccgagaacaattacaagaccacaccacccgtgctggactctgatggctccttctttctgtattctaggctgacagtggataagtcccggtggcaggagggcaacgtgtttagctgctctgtgatgcacgaggccctgcacaatcattatacccagaagtccctgagcctgtctctgggcaagtga

SEQ ID NO: 163 - protein, 219 aa, 人工序列(Artificial Sequence); identical to SEQ ID NO: 159

SEQ ID NO: 164 - DNA, 660 bp, 人工序列(Artificial Sequence); identical to SEQ ID NO: 160

SEQ ID NO: 165 - protein, 446 aa, 人工序列(Artificial Sequence)
QVQLVQSGAEVKKPGASVKVSCKASGYTFTNYGMNWVRQAPGQGLKWMGWINTNTGEPTYAQELQGRVTMTLDTSTRTAYMELRSLRSDDTAVYYCARFSHLRGPMDYWGQGTLVTVSSASTKGPSVFPLAPCSRSTSESTAALGCLVKDYFPEPVTVSWNSGALTSGVHTFPAVLQSSGLYSLSSVVTVPSSSLGTKTYTCNVDHKPSNTKVDKRVESKYGPPCPPCPAPEFLGGPSVFLFPPKPKDTLMISRTPEVTCVVVDVSQEDPEVQFNWYVDGVEVHNAKTKPREEQFNSTYRVVSVLTVLHQDWLNGKEYKCKVSNKGLPSSIEKTISKAKGQPREPQVYTLPPSQEEMTKNQVSLTCLVKGFYPSDIAVEWESNGQPENNYKTTPPVLDSDGSFFLYSRLTVDKSRWQEGNVFSCSVMHEALHNHYTQKSLSLSLGK

SEQ ID NO: 166 - DNA, 1341 bp, 人工序列(Artificial Sequence)
caggtgcagctggtgcagtccggagctgaggtgaagaagccaggagctagcgtgaaggtgtcttgcaaggcctccggctacaccttcacaaactatggcatgaattgggtgaggcaggctccaggacagggcctgaagtggatgggatggatcaacaccaatacaggcgagcctacatacgcccaggagctgcagggcagggtgaccatgacactggacaccagcacaagaaccgcttatatggagctgaggtctctgcggtccgacgataccgccgtgtactattgtgctagattttctcacctgaggggaccaatggattactggggacagggcacactggtgaccgtgtccagcgcctctacaaagggcccttccgtgttcccactggctccctgctccagaagcacatctgagtccaccgccgctctgggctgtctggtgaaggactacttccctgagccagtgaccgtgtcctggaacagcggcgccctgacatctggcgtgcacacctttccagctgtgctgcagtccagcggcctgtactccctgtcttccgtggtgacagtgcccagctcttccctgggcaccaagacatatacctgcaacgtggaccataagccttccaataccaaggtggataagagggtggagagcaagtacggaccaccttgcccaccatgtccagctcctgagtttctgggaggaccatccgtgttcctgtttcctccaaagcctaaggacaccctgatgatcagccggacacctgaggtgacctgcgtggtggtggacgtgtctcaggaggatccagaggtgcagttcaactggtacgtggatggcgtggaggtgcacaatgctaagaccaagccaagagaggagcagtttaattccacataccgcgtggtgagcgtgctgaccgtgctgcatcaggattggctgaacggcaaggagtataagtgcaaggtgtccaataagggcctgcccagctctatcgagaagacaatcagcaaggctaagggacagcctagggagccacaggtgtacaccctgcccccttctcaggaggagatgacaaagaaccaggtgtccctgacctgtctggtgaagggcttctatccaagcgacatcgctgtggagtgggagtctaatggccagcccgagaacaattacaagaccacaccacccgtgctggactctgatggctccttctttctgtattctaggctgacagtggataagtcccggtggcaggagggcaacgtgtttagctgctctgtgatgcacgaggccctgcacaatcattatacccagaagtccctgagcctgtctctgggcaagtga

SEQ ID NO: 167 - protein, 219 aa, 人工序列(Artificial Sequence); identical to SEQ ID NO: 159

SEQ ID NO: 168 - DNA, 660 bp, 人工序列(Artificial Sequence); identical to SEQ ID NO: 160

SEQ ID NO: 169 - protein, 446 aa, 人工序列(Artificial Sequence); identical to SEQ ID NO: 165

SEQ ID NO: 170 - DNA, 1341 bp, 人工序列(Artificial Sequence); identical to SEQ ID NO: 166

SEQ ID NO: 171 - protein, 219 aa, 人工序列(Artificial Sequence)
DAQMTQSPSSLSASVGDRVTITCRSSQSLVHSNGYTYLHWYQQKPGKAPKLLIYKVSNRFSGVPSRFSGSGSGTDFTLTISSLQPEDFATYYCSQSTHVPPTFGQGTKLEIKRTVAAPSVFIFPPSDEQLKSGTASVVCLLNNFYPREAKVQWKVDNALQSGNSQESVTEQDSKDSTYSLSSTLTLSKADYEKHKVYACEVTHQGLSSPVTKSFNRGEC

SEQ ID NO: 172 - DNA, 660 bp, 人工序列(Artificial Sequence)
gacgcccagatgacacagtccccatccagcctgtccgctagcgtgggcgatagggtgaccatcacatgccggtcttcccagagcctggtgcactctaacggctacacctatctgcattggtaccagcagaagccaggcaaggcccccaagctgctgatctataaggtgtccaatagattcagcggcgtgccttctcgcttttctggctccggcagcggcacagacttcaccctgacaatcagctctctgcagccagaggattttgctacctactattgttctcagtccacccacgtgccccctacattcggccagggcaccaagctggagatcaagcgtacggtggccgctcccagcgtgttcatctttcccccttctgacgagcagctgaagtctggcaccgcttccgtggtgtgcctgctgaacaatttctaccccagagaggccaaggtgcagtggaaggtggataacgctctgcagtccggcaatagccaggagtctgtgaccgagcaggactccaaggatagcacatattctctgtcttccaccctgacactgtctaaggccgactacgagaagcacaaggtgtatgcttgcgaggtgacccatcagggcctgagctctcctgtgacaaagtcctttaatcgcggcgagtgttga

SEQ ID NO: 173 - protein, 446 aa, 人工序列(Artificial Sequence); identical to SEQ ID NO: 157

SEQ ID NO: 174 - DNA, 1341 bp, 人工序列(Artificial Sequence); identical to SEQ ID NO: 158

SEQ ID NO: 175 - protein, 219 aa, 人工序列(Artificial Sequence); identical to SEQ ID NO: 171

SEQ ID NO: 176 - DNA, 660 bp, 人工序列(Artificial Sequence); identical to SEQ ID NO: 172

SEQ ID NO: 177 - protein, 446 aa, 人工序列(Artificial Sequence); identical to SEQ ID NO: 161

SEQ ID NO: 178 - DNA, 1341 bp, 人工序列(Artificial Sequence); identical to SEQ ID NO: 162

SEQ ID NO: 179 - protein, 219 aa, 人工序列(Artificial Sequence); identical to SEQ ID NO: 171

SEQ ID NO: 180 - DNA, 660 bp, 人工序列(Artificial Sequence); identical to SEQ ID NO: 172

SEQ ID NO: 181 - protein, 447 aa, 人工序列(Artificial Sequence)
QVQLVQSGAEVKKPGASVKVSCKVSGFNIEDDYIEWVRQAPGQGLEWMGRIDPANDKTKYAQKFQGRVTMTGDTSTNTVYMELSSLRSEDTAVYYCARPGLRRYYSMDYWGQGTLVTVSSASTKGPSVFPLAPCSRSTSESTAALGCLVKDYFPEPVTVSWNSGALTSGVHTFPAVLQSSGLYSLSSVVTVPSSSLGTKTYTCNVDHKPSNTKVDKRVESKYGPPCPPCPAPEFLGGPSVFLFPPKPKDTLMISRTPEVTCVVVDVSQEDPEVQFNWYVDGVEVHNAKTKPREEQFNSTYRVVSVLTVLHQDWLNGKEYKCKVSNKGLPSSIEKTISKAKGQPREPQVYTLPPSQEEMTKNQVSLTCLVKGFYPSDIAVEWESNGQPENNYKTTPPVLDSDGSFFLYSRLTVDKSRWQEGNVFSCSVMHEALHNHYTQKSLSLSLGK

SEQ ID NO: 182 - DNA, 1344 bp, 人工序列(Artificial Sequence)
caggtgcagctggtgcagtccggagctgaggtgaagaagccaggagctagcgtgaaggtgtcttgcaaggtgtccggcttcaacatcgaggacgattacatcgagtgggtgaggcaggctccaggacagggactggagtggatgggaaggatcgaccctgccaacgataagacaaagtacgctcagaagtttcagggcagagtgaccatgacaggcgacaccagcacaaataccgtgtatatggagctgtccagcctgcgctctgaggataccgccgtgtactattgtgctaggcccggcctgagacgctactattccatggactattggggccagggcacactggtgaccgtgtcttccgcctctacaaagggcccttccgtgttcccactggctccctgctccagaagcacatctgagtccaccgccgctctgggctgtctggtgaaggactacttccctgagccagtgaccgtgtcctggaacagcggcgccctgacatctggcgtgcacacctttccagctgtgctgcagtccagcggcctgtactccctgtcttccgtggtgacagtgcccagctcttccctgggcaccaagacatatacctgcaacgtggaccataagccttccaataccaaggtggataagagggtggagagcaagtacggaccaccttgcccaccatgtccagctcctgagtttctgggaggaccatccgtgttcctgtttcctccaaagcctaaggacaccctgatgatcagccggacacctgaggtgacctgcgtggtggtggacgtgtctcaggaggatccagaggtgcagttcaactggtacgtggatggcgtggaggtgcacaatgctaagaccaagccaagagaggagcagtttaattccacataccgcgtggtgagcgtgctgaccgtgctgcatcaggattggctgaacggcaaggagtataagtgcaaggtgtccaataagggcctgcccagctctatcgagaagacaatcagcaaggctaagggacagcctagggagccacaggtgtacaccctgcccccttctcaggaggagatgacaaagaaccaggtgtccctgacctgtctggtgaagggcttctatccaagcgacatcgctgtggagtgggagtctaatggccagcccgagaacaattacaagaccacaccacccgtgctggactctgatggctccttctttctgtattctaggctgacagtggataagtcccggtggcaggagggcaacgtgtttagctgctctgtgatgcacgaggccctgcacaatcattatacccagaagtccctgagcctgtctctgggcaagtga

SEQ ID NO: 183 - protein, 214 aa, 人工序列(Artificial Sequence)
DIQMTQSPSSLSASVGDRVTITCKASENVVSYVSWYQQKPGKAPKLLIYGASNRYTGVPSRFIGSGSSTDFTLTISSLQPEDFATYYCGQSYSYPLTFGQGTKLEIKRTVAAPSVFIFPPSDEQLKSGTASVVCLLNNFYPREAKVQWKVDNALQSGNSQESVTEQDSKDSTYSLSSTLTLSKADYEKHKVYACEVTHQGLSSPVTKSFNRGEC

SEQ ID NO: 184 - DNA, 645 bp, 人工序列(Artificial Sequence)
gacatccagatgacccagagcccttccagcctgtccgccagcgtgggcgatagggtgaccatcacatgcaaggcttctgagaacgtggtgtcctacgtgagctggtatcagcagaagcccggcaaggcccctaagctgctgatctacggcgcttctaataggtataccggagtgccatcccggttcatcggatccggctcttccacagactttaccctgacaatcagctctctgcagccagaggatttcgccacatactattgtggccagagctactcttatcccctgacctttggccagggcacaaagctggagatcaagcgtacggtggccgctcccagcgtgttcatctttcccccttctgacgagcagctgaagtctggcaccgcttccgtggtgtgcctgctgaacaatttctaccccagagaggccaaggtgcagtggaaggtggataacgctctgcagtccggcaatagccaggagtctgtgaccgagcaggactccaaggatagcacatattctctgtcttccaccctgacactgtctaaggccgactacgagaagcacaaggtgtatgcttgcgaggtgacccatcagggcctgagctctcctgtgacaaagtcctttaatcgcggcgagtgttga

SEQ ID NO: 185 - protein, 447 aa, 人工序列(Artificial Sequence)
QVQLVQSGAEVKKPGASVKVSCKVSGFNIEDDYIEWVRQAPGQGLEWMGRIDPANDKTKYAQKFQGRVTMTGDTSTNTVYMELSSLRSEDTAVYYCTRPGLRRYYSMDYWGQGTLVTVSSASTKGPSVFPLAPCSRSTSESTAALGCLVKDYFPEPVTVSWNSGALTSGVHTFPAVLQSSGLYSLSSVVTVPSSSLGTKTYTCNVDHKPSNTKVDKRVESKYGPPCPPCPAPEFLGGPSVFLFPPKPKDTLMISRTPEVTCVVVDVSQEDPEVQFNWYVDGVEVHNAKTKPREEQFNSTYRVVSVLTVLHQDWLNGKEYKCKVSNKGLPSSIEKTISKAKGQPREPQVYTLPPSQEEMTKNQVSLTCLVKGFYPSDIAVEWESNGQPENNYKTTPPVLDSDGSFFLYSRLTVDKSRWQEGNVFSCSVMHEALHNHYTQKSLSLSLGK

SEQ ID NO: 186 - DNA, 1344 bp, 人工序列(Artificial Sequence)
caggtgcagctggtgcagtccggagctgaggtgaagaagccaggagctagcgtgaaggtgtcttgcaaggtgtccggcttcaacatcgaggacgattacatcgagtgggtgaggcaggctccaggacagggactggagtggatgggaaggatcgaccctgccaacgataagacaaagtacgctcagaagtttcagggcagagtgaccatgacaggcgacaccagcacaaataccgtgtatatggagctgtccagcctgcgctctgaggatacagccgtgtactattgtaccaggcccggcctgagacgctactattccatggactattggggccagggcacactggtgaccgtgtcttccgcctctacaaagggcccttccgtgttcccactggctccctgctccagaagcacatctgagtccaccgccgctctgggctgtctggtgaaggactacttccctgagccagtgaccgtgtcctggaacagcggcgccctgacatctggcgtgcacacctttccagctgtgctgcagtccagcggcctgtactccctgtcttccgtggtgacagtgcccagctcttccctgggcaccaagacatatacctgcaacgtggaccataagccttccaataccaaggtggataagagggtggagagcaagtacggaccaccttgcccaccatgtccagctcctgagtttctgggaggaccatccgtgttcctgtttcctccaaagcctaaggacaccctgatgatcagccggacacctgaggtgacctgcgtggtggtggacgtgtctcaggaggatccagaggtgcagttcaactggtacgtggatggcgtggaggtgcacaatgctaagaccaagccaagagaggagcagtttaattccacataccgcgtggtgagcgtgctgaccgtgctgcatcaggattggctgaacggcaaggagtataagtgcaaggtgtccaataagggcctgcccagctctatcgagaagacaatcagcaaggctaagggacagcctagggagccacaggtgtacaccctgcccccttctcaggaggagatgacaaagaaccaggtgtccctgacctgtctggtgaagggcttctatccaagcgacatcgctgtggagtgggagtctaatggccagcccgagaacaattacaagaccacaccacccgtgctggactctgatggctccttctttctgtattctaggctgacagtggataagtcccggtggcaggagggcaacgtgtttagctgctctgtgatgcacgaggccctgcacaatcattatacccagaagtccctgagcctgtctctgggcaagtga

SEQ ID NO: 187 - protein, 214 aa, 人工序列(Artificial Sequence); identical to SEQ ID NO: 183

SEQ ID NO: 188 - DNA, 645 bp, 人工序列(Artificial Sequence); identical to SEQ ID NO: 184

SEQ ID NO: 189 - DNA, 348 bp, Mus musculus
caggtgcagctgaaggagtctggaccaggactggtggctccatctcagtccctgagcatcacctgcacagtgtccggcttcagcctgaccaactacggagtgcactgggtgaggcagccacctggcaagggactggagtggctgggcatcatctgggctggcggctccacaaactataattctgccctgatgtcccggctgtctatctccaaggacaacagcaagtctcaggtgtttctgaagatgaatagcctgcagaccgacgatacagccatgtactattgtgctagggacgattacgccagcatggattattggggccagggcacctctgtgacagtgtccagc

SEQ ID NO: 190 - DNA, 336 bp, Mus musculus
gacgccttcatgacccagacaccactgtccctgcctgtgagcctgggcgatcaggcttctatctcctgcagatccagccagtctctggtgcactccaacggcaatacatacctgcattggtatctgcagaagccaggccagtcccccaagctgctgatctacaaggtgagcaacaggttctctggcgtgcctgaccggtttagcggctctggctccggcaccgatttcacactgaagatctccagggtggaggctgaggacctgggcgtgtacttttgtagccagtctacccacgtgccatatacactgggcggcggcaccaagctggagatcaag

SEQ ID NO: 191 - DNA, 357 bp, Mus musculus
gaggtgcagctgcagcagtctggccccgagctgaagaagcctggcgagaccgtgaagatctcttgcaaggcctccggctacaccttcacaaactatggcatgaattgggtgaagcaggtgccaggcaagggcctgaagtggatgggctggatcaacaccaatacaggcgagcccacatacgccgaggagttcaagggcagattcgcttttagcctggagacctctgcccgcacagcttttctgcagatcaacaatctgaagaacgaggacaccgccacatacttctgtaccaggttttcccacctgcggggccccatggattattggggccagggcgctagcgtgacagtgtccagc

SEQ ID NO: 192 - DNA, 336 bp, Mus musculus
gacgccgtgatgacccagacaccactgtccctgcccgtgagcctgggcgatcaggcttctatctcctgcagatccagccagtctctggtgcactccaacggctacacatatctgcattggtacctgcagaagcctggccagtccccaaagctgctgatctataaggtgagcaataggttctctggagtgccagaccggtttagcggatctggatccggcaccgatttcacactgaagatctccaggctggaggctgaggacctgggcgtgtacttctgtagccagtctacccacgtgccccctacatttggcggcggcaccaagctggagatcaag

SEQ ID NO: 193 - DNA, 336 bp, Mus musculus
gaagtgatgctggtggagagcggaggaggactggtgcagccaggaggcagcctgaagctgtcttgcgccgcttccggcttcacctttagcaactactatatgtcttgggtgagacagacacccgagaagcgcctggagtgggtggcttacatctccagcggaggaggatccacctactatcctgacagcgtgaagggcaggttcaccatctctcgggataacgccaagaatacactgtacctgcagatgtcttccctgaagtccgaggacacagctatgtactattgtgcctggtttgcttattggggccagggcaccctggtgacagtgtctgct

SEQ ID NO: 194 - DNA, 336 bp, Mus musculus
gacgccgtggtgacccagacaccactgaccctgtccgtgacaatcggccagcccgcttctatctcctgcaagtccagccagtccctgctggacagcgatggcaagacatacctgaactggctgctgcagaggccaggacagagccctaagcggctgatctatctggtgtctaagctggactccggcgtgcctgatagattcaccggcagcggctctggcaccgactttacactgaagatctctcgcgtggaggccgaggatctgggcgtgtactattgttggcagggcacccacttcccactgacatttggcgctggcaccaagctggagctgaag

SEQ ID NO: 195 - DNA, 351 bp, Mus musculus
gaggtgcagctgcagcagtctgtggccgagctgatgaagccaggcgcttccgtgaagatctactgcaaggccaccggctacacattcagcagatattggatcgagtgggtgaagcagaggccaggacacggactggagtggatcggcgagttcatccctggctctgacaccacaaacttcaatgagaagtttaagggcaaggccacctttacagctgagatctccagcaacaccgcttatatgcagctgtcttccctgacatccgaggacagcgccgtgtacttttgtgctaggggcggcctgaggcggatggattattggggccagggcacctccgtgacagtgagctct

SEQ ID NO: 196 - DNA, 324 bp, Mus musculus
gacatcgtgatgacccagacacccgccatcatgtccgcctctcctggcgagaaggtgaccatgacatgcagggcctccagctccgtgtccagcacctacctgcactggtatcagcagaagagcggcgcttctccaaagctgtggatctacaccacatccacactggctagcggagtgccagctcggttctccggaagcggatctggcacctcctatagcctgacaatctcttccgtggaggccgaggacgccgctacctactattgtcagcagttctctgattccacctggacatttggcggcggcacaaagctggagatcaag

SEQ ID NO: 197 - DNA, 360 bp, Mus musculus
gaggtgcagctgcagcagtctggagctgaggtggctaggccaggagcttccgtgaagctgagctgcaccgtgtctggcttcaacatcgaggacgattacatcgagtgggtgaagcagagaccagagcagggactggagtggatcggaaggatcgaccccgccaacgataagacaaagtacgctcctaagtttcaggacaaggccaccatcacaggcgatacctccagcaatacagcttatctgcagctgtcttccctgacctccgaggacacagccgtgtactattgtaccagacccggcctgaggcggtactattccatggattattggggccagggcaccagcgtgacagtgagctct

SEQ ID NO: 198 - DNA, 321 bp, Mus musculus
aacatcgtgctgacccagtcccctaagagcatgtctatgtccgtgggcgagagggtgacactgtcttgcaaggcctccgagaacgtggtgtcctacgtgagctggtatcagcagaagcccgagcagagccctaagctgctgatctacggcgcttctaataggtataccggagtgccagaccggttcatcggatccggctccagcaccgatttcacactgatcatctcttcctttcagccagaggacctggccgattaccactgtggccagagctactcttatcccctgacctttggcgctggcacaaagctggagctgaag